European Patent Application EP 4 488 389 A1, published January 8, 2025. Title: Signature for the prognosis of brain metastasis relapse after brain surgery. Applicant: Fundación del Sector Público Estatal Centro Nacional de Investigaciones Oncológicas Carlos III (F.S.P. CNIO). Application EP. The sequence listing filed with the application follows.

SEQUENCE LISTING (10 sequences)

SEQ ID NO: 1 - DNA, 20 bp, Synthetic construct
  source 1..20: mol_type = other DNA
agcttggactctttgggctc

SEQ ID NO: 2 - DNA, 20 bp, Synthetic construct
  source 1..20: mol_type = other DNA
gcagtctttggctcaacagc

SEQ ID NO: 3 - DNA, 20 bp, Synthetic construct
  source 1..20: mol_type = other DNA
cagccaaaccaattgccctc

SEQ ID NO: 4 - DNA, 20 bp, Synthetic construct
  source 1..20: mol_type = other DNA
ggggtggggatgtcacaaat

SEQ ID NO: 5 - DNA, 20 bp, Synthetic construct
  source 1..20: mol_type = other DNA
cactgtgccttgtgtttggg

SEQ ID NO: 6 - DNA, 20 bp, Synthetic construct
  source 1..20: mol_type = other DNA
ggccactgctaggtttctca

SEQ ID NO: 7 - DNA, 20 bp, Synthetic construct
  source 1..20: mol_type = other DNA
aacgtaccggccactatcac

SEQ ID NO: 8 - DNA, 20 bp, Synthetic construct
  source 1..20: mol_type = other DNA
tggtagcccaagacagaggt

SEQ ID NO: 9 - DNA, 20 bp, Synthetic construct
  source 1..20: mol_type = other DNA
cctccccttgtgtcaactcc

SEQ ID NO: 10 - DNA, 19 bp, Synthetic construct
  source 1..19: mol_type = other DNA
gtggctccggtgatttggg